European Patent Application EP 4 471 122 A1, published December 4, 2024. Title: RECOMBINANT MICROORGANISM, METHOD FOR CONSTRUCTING SAME AND USE THEREOF. Applicant: Langfang Meihua Biotechnology Development Co.,Ltd. Application EP 22923640.1, filed December 28, 2022. The sequence listing filed with the application follows.

SEQUENCE LISTING (51 sequences)

SEQ ID NO: 1 - DNA, 192 bp, synthetic construct
  source 1..192: mol_type = other DNA
tagctgccaattattccgggcttgtgacccgctacccgataaataggtcggctgaaaaatttcgttgcaatatcaacaaaaaggcctatcattgggaggtgtcgcaccaagtacttttgcgaagcgccatctgacggattttcaaaagatgtatatgctcggtgcggaaacctacgaaaggattttttaccc

SEQ ID NO: 2 - DNA, 260 bp, synthetic construct
  source 1..260: mol_type = other DNA
acctgcgtttataaagaaatgtaaacgtgatcggatcgatataaaagaaacagtttgtactcaggtttgaagcattttctccaattcgcctggcaaaaatctcaattgtcgcttacagtttttctcaacgacaggctgctaagctgctagttcggtggcctagtgagtggcgtttacttggataaaagtaatcccatgtcgtgatcagccattttgggttgtttccatagcatccaaaggtttcgtctttcgatacctat

SEQ ID NO: 3 - DNA, 46 bp, synthetic construct
  source 1..46: mol_type = other DNA
aattcgagctcggtacccggggatcctgacagttgctgatctggct

SEQ ID NO: 4 - DNA, 40 bp, synthetic construct
  source 1..40: mol_type = other DNA
cccggaataattggcagctatagagtaattattcctttca

SEQ ID NO: 5 - DNA, 40 bp, synthetic construct
  source 1..40: mol_type = other DNA
tgaaaggaataattactctatagctgccaattattccggg

SEQ ID NO: 6 - DNA, 40 bp, synthetic construct
  source 1..40: mol_type = other DNA
gaagatgtgtgagtcgacacgggtaaaaaatcctttcgta

SEQ ID NO: 7 - DNA, 40 bp, synthetic construct
  source 1..40: mol_type = other DNA
tacgaaaggattttttacccgtgtcgactcacacatcttc

SEQ ID NO: 8 - DNA, 43 bp, synthetic construct
  source 1..43: mol_type = other DNA
ggtggagcctgaaggaggtgcgagtgatcggcaatgaatccgg

SEQ ID NO: 9 - DNA, 43 bp, synthetic construct
  source 1..43: mol_type = other DNA
ccggattcattgccgatcactcgcacctccttcaggctccacc

SEQ ID NO: 10 - DNA, 46 bp, synthetic construct
  source 1..46: mol_type = other DNA
gtaaaacgacggccagtgccaagcttcgcggcagacggagtctggg

SEQ ID NO: 11 - DNA, 46 bp, synthetic construct
  source 1..46: mol_type = other DNA
aattcgagctcggtacccggggatccagcgacaggacaagcactgg

SEQ ID NO: 12 - DNA, 40 bp, synthetic construct
  source 1..40: mol_type = other DNA
cccggaataattggcagctatgtgcacctttcgatctacg

SEQ ID NO: 13 - DNA, 40 bp, synthetic construct
  source 1..40: mol_type = other DNA
cgtagatcgaaaggtgcacatagctgccaattattccggg

SEQ ID NO: 14 - DNA, 41 bp, synthetic construct
  source 1..41: mol_type = other DNA
tttctgtacgaccagggccatgggtaaaaaatcctttcgta

SEQ ID NO: 15 - DNA, 41 bp, synthetic construct
  source 1..41: mol_type = other DNA
tacgaaaggattttttacccatggccctggtcgtacagaaa

SEQ ID NO: 16 - DNA, 42 bp, synthetic construct
  source 1..42: mol_type = other DNA
tcggaacgagggcaggtgaaggtgatgtcggtggtgccgtct

SEQ ID NO: 17 - DNA, 42 bp, synthetic construct
  source 1..42: mol_type = other DNA
agacggcaccaccgacatcaccttcacctgccctcgttccga

SEQ ID NO: 18 - DNA, 46 bp, synthetic construct
  source 1..46: mol_type = other DNA
gtaaaacgacggccagtgccaagcttagcctggtaagaggaaacgt

SEQ ID NO: 19 - DNA, 46 bp, synthetic construct
  source 1..46: mol_type = other DNA
aattcgagctcggtacccggggatccctgcgggcagatccttttga

SEQ ID NO: 20 - DNA, 40 bp, synthetic construct
  source 1..40: mol_type = other DNA
atttctttataaacgcaggtcatatctaccaaaactacgc

SEQ ID NO: 21 - DNA, 40 bp, synthetic construct
  source 1..40: mol_type = other DNA
gcgtagttttggtagatatgacctgcgtttataaagaaat

SEQ ID NO: 22 - DNA, 40 bp, synthetic construct
  source 1..40: mol_type = other DNA
gtatatctccttctgcaggaataggtatcgaaagacgaaa

SEQ ID NO: 23 - DNA, 40 bp, synthetic construct
  source 1..40: mol_type = other DNA
tttcgtctttcgatacctattcctgcagaaggagatatac

SEQ ID NO: 24 - DNA, 41 bp, synthetic construct
  source 1..41: mol_type = other DNA
tagccaattcagccaaaacccccacgcgatcttccacatcc

SEQ ID NO: 25 - DNA, 41 bp, synthetic construct
  source 1..41: mol_type = other DNA
ggatgtggaagatcgcgtgggggttttggctgaattggcta

SEQ ID NO: 26 - DNA, 46 bp, synthetic construct
  source 1..46: mol_type = other DNA
gtaaaacgacggccagtgccaagcttgctggctcttgccgtcgata

SEQ ID NO: 27 - DNA, 46 bp, synthetic construct
  source 1..46: mol_type = other DNA
attcgagctcggtacccggggatccgccgttgatcattgttcttca

SEQ ID NO: 28 - DNA, 40 bp, synthetic construct
  source 1..40: mol_type = other DNA
cccggaataattggcagctaggatataaccctatcccaag

SEQ ID NO: 29 - DNA, 40 bp, synthetic construct
  source 1..40: mol_type = other DNA
cttgggatagggttatatcctagctgccaattattccggg

SEQ ID NO: 30 - DNA, 41 bp, synthetic construct
  source 1..41: mol_type = other DNA
acgcgtcgaaatgtagtccatgggtaaaaaatcctttcgta

SEQ ID NO: 31 - DNA, 41 bp, synthetic construct
  source 1..41: mol_type = other DNA
tacgaaaggattttttacccatggactacatttcgacgcgt

SEQ ID NO: 32 - DNA, 46 bp, synthetic construct
  source 1..46: mol_type = other DNA
gtaaaacgacggccagtgccaagcttgaatacgcggattccctcgc

SEQ ID NO: 33 - DNA, 38 bp, synthetic construct
  source 1..38: mol_type = other DNA
agctcggtacccggggatcctgtccaactgcggtgatt

SEQ ID NO: 34 - DNA, 40 bp, synthetic construct
  source 1..40: mol_type = other DNA
ggtagacaagcaaggcaacaggcaaatgtgtttatcttcc

SEQ ID NO: 35 - DNA, 40 bp, synthetic construct
  source 1..40: mol_type = other DNA
ggaagataaacacatttgcctgttgccttgcttgtctacc

SEQ ID NO: 36 - DNA, 38 bp, synthetic construct
  source 1..38: mol_type = other DNA
caatacggagcggttacaaagcttggcactggccgtcg

SEQ ID NO: 37 - DNA, 55 bp, synthetic construct
  source 1..55: mol_type = other DNA
catgattacgaattcgagctcggtacccggggatcccgtgcgtggattgtcagca

SEQ ID NO: 38 - DNA, 40 bp, synthetic construct
  source 1..40: mol_type = other DNA
gatcacgctatagttgcgccgtgggaaagacatatgtggg

SEQ ID NO: 39 - DNA, 40 bp, synthetic construct
  source 1..40: mol_type = other DNA
cccacatatgtctttcccacggcgcaactatagcgtgatc

SEQ ID NO: 40 - DNA, 57 bp, synthetic construct
  source 1..57: mol_type = other DNA
tcacgacgttgtaaaacgacggccagtgccaagcttcacggtcgggatttctaacag

SEQ ID NO: 41 - DNA, 57 bp, synthetic construct
  source 1..57: mol_type = other DNA
catgattacgaattcgagctcggtacccggggatccagtagacacctcgaacgctac

SEQ ID NO: 42 - DNA, 42 bp, synthetic construct
  source 1..42: mol_type = other DNA
gatcacgctatagttgcgccgaaaaggagcttgctttacgac

SEQ ID NO: 43 - DNA, 42 bp, synthetic construct
  source 1..42: mol_type = other DNA
gtcgtaaagcaagctccttttcggcgcaactatagcgtgatc

SEQ ID NO: 44 - DNA, 57 bp, synthetic construct; identical to SEQ ID NO: 40
  source 1..57: mol_type = other DNA

SEQ ID NO: 45 - DNA, 52 bp, synthetic construct
  source 1..52: mol_type = other DNA
cgagctcggtacccggggatccacccgggtgtggcgcgcaagaagatgccag

SEQ ID NO: 46 - DNA, 46 bp, synthetic construct
  source 1..46: mol_type = other DNA
taaatgttgtacgcggaccagaacaagattccgccgtggaccacgc

SEQ ID NO: 47 - DNA, 43 bp, synthetic construct
  source 1..43: mol_type = other DNA
ggcggaatcttgttctggtccgcgtacaacatttacatacacc

SEQ ID NO: 48 - DNA, 51 bp, synthetic construct
  source 1..51: mol_type = other DNA
gtaaaacgacggccagtgccaagcttagcaaggtgttagagcaaattttcg

SEQ ID NO: 49 - DNA, 47 bp, synthetic construct
  source 1..47: mol_type = other DNA
gaattcgagctcggtacccggggatccaacttgtaaccgctccgtat

SEQ ID NO: 50 - DNA, 48 bp, synthetic construct
  source 1..48: mol_type = other DNA
ggtgtatgtaaatgttgtacgcggaccagtgcttgccttgcttgtcta

SEQ ID NO: 51 - DNA, 48 bp, synthetic construct
  source 1..48: mol_type = other DNA
tagacaagcaaggcaagcactggtccgcgtacaacatttacatacacc